European Patent Application EP 4 711 764 A2, published March 18, 2026. Title: Systems and methods for biomolecule quantitation. Applicant: Nautilus Subsidiary, Inc. The sequence listing filed with the application follows.

SEQUENCE LISTING (2 sequences)

SEQ ID NO: 1 - DNA, 20 bp, synthetic construct
  misc_feature 1..20: note = Exemplary aptamer
  source 1..20: mol_type = other DNA
gcggttgaaggcccgaccgt

SEQ ID NO: 2 - protein, 5 aa, synthetic construct
  REGION 1..5: note = Synthetic Peptide
YKACP